European Patent Specification EP 3 597 738 B1, published April 5, 2023. Title: Modified homoserine dehydrogenase and method for producing homoserine or L-amino acid derived from homoserine using the same. Applicant: CJ CheilJedang Corporation. The sequence listing filed with the application follows.

SEQUENCE LISTING (50 sequences)

SEQ ID NO: 1 - protein, 445 aa, Artificial Sequence
  homoserine dehydrogenase
MTSASAPSFNPGKGPGSAVGIALLGFGTVGTEVMRLMTEYGDELAHRIGGPLEVRGIAVSDISKPREGVAPELLTEDAFALIEREDVDIVVEVIGGIEYPREVVLAALKAGKSVVTANKALVAAHSAELADAAEAANVDLYFEAAVAGAIPVVGPLRRSLAGDQIQSVMGIVNGTTNFILDAMDSTGADYADSLAEATRLGYAEADPTADVEGHDAASKAAILASIAFHTRVTADDVYCEGISNISAADIEAAQQAGHTIKLLAICEKFTNKEGKSAISARVHPTLLPVSHPLASVNKSFNAIFVEAEAAGRLMFYGNGAGGAPTASAVLGDVVGAARNKVHGGRAPGESTYANLPIADFGETTTRYHLDMDVEDRVGVLAELASLFSEQGISLRTIRQEERDDDARLIVVTHSALESDLSRTVELLKAKPVVKAINSVIRLERD

SEQ ID NO: 2 - DNA, 930 bp, Artificial Sequence
  thrB gene
atggcaattgaactgaacgtcggtcgtaaggttaccgtcacggtacctggatcttctgcaaacctcggacctggctttgacactttaggtttggcactgtcggtatacgacactgtcgaagtggaaattattccatctggcttggaagtggaagtttttggcgaaggccaaggcgaagtccctcttgatggctcccacctggtggttaaagctattcgtgctggcctgaaggcagctgacgctgaagttcctggattgcgagtggtgtgccacaacaacattccgcagtctcgtggtcttggctcctctgctgcagcggcggttgctggtgttgctgcagctaatggtttggcggatttcccgctgactcaagagcagattgttcagttgtcctctgcctttgaaggccacccagataatgctgcggcttctgtgctgggtggagcagtggtgtcgtggacaaatctgtctatcgacggcaagagccagccacagtatgctgctgtaccacttgaggtgcaggacaatattcgtgcgactgcgctggttcctaatttccacgcatccaccgaagctgtgcgccgagtccttcccactgaagtcactcacatcgatgcgcgatttaacgtgtcccgcgttgcagtgatgatcgttgcgttgcagcagcgtcctgatttgctgtgggagggtactcgtgaccgtctgcaccagccttatcgtgcagaagtgttgcctattacctctgagtgggtaaaccgcctgcgcaaccgtggctacgcggcatacctttccggtgccggcccaaccgccatggtgctgtccactgagccaattccagacaaggttttggaagatgctcgtgagtctggcattaaggtgcttgagcttgaggttgcgggaccagtcaaggttgaagttaaccaaccttag

SEQ ID NO: 3 - DNA, 18 bp, Artificial Sequence
  primer
ctgcgacagcatggaact

SEQ ID NO: 4 - DNA, 18 bp, Artificial Sequence
  primer
caacgacaaacgcccatc

SEQ ID NO: 5 - DNA, 2778 bp, Artificial Sequence
  gene fragment
ctgcgacagcatggaactcagtgcaatggctgtaaggcctgcaccaacaatgattgagcgaagctccaaaatgtcctccccgggttgatattagatttcataaatatactaaaaatcttgagagtttttccgttgaaaactaaaaagctgggaaggtgaatcgaatttcggggctttaaagcaaaaatgaacagcttggtctatagtggctaggtaccctttttgttttggacacatgtagggtggccgaaacaaagtaataggacaacaacgctcgaccgcgattatttttggagaatcatgacctcagcatctgccccaagctttaaccccggcaagggtcccggctcagcagtcggaattgcccttttaggattcggaacagtcggcactgaggtgatgcgtctgatgaccgagtacggtgatgaacttgcgcaccgcattggtggcccactggaggttcgtggcattgctgtttctgatatctcaaagccacgtgaaggcgttgcacctgagctgctcactgaggacgcttttgcactcatcgagcgcgaggatgttgacatcgtcgttgaggttatcggcggcattgagtacccacgtgaggtagttctcgcagctctgaaggccggcaagtctgttgttaccgccaataaggctcttgttgcagctcactctgctgagcttgctgatgcagcggaagccgcaaacgttgacctgtacttcgaggctgctgttgcaggcgcaattccagtggttggcccactgcgtcgctccctggctggcgatcagatccagtctgtgatgggcatcgttaacggcaccaccaacttcatcttggacgccatggattccaccggcgctgactatgcagattctttggctgaggcaactcgtttgggttacgccgaagctgatccaactgcagacgtcgaaggccatgacgccgcatccaaggctgcaattttggcatccatcgctttccacacccgtgttaccgcggatgatgtgtactgcgaaggtatcagcaacatcagcgctgccgacattgaggcagcacagcaggcaggccacaccatcaagttgttggccatctgtgagaagttcaccaacaaggaaggaaagtcggctatttctgctcgcgtgcacccgactctattacctgtgtcccacccactggcgtcggtaaacaagtcctttaatgcaatctttgttgaagcagaagcagctggtcgcctgatgttctacggaaacggtgcaggtggcgcgccaaccgcgtctgctgtgcttggcgacgtcgttggtgccgcacgaaacaaggtgcacggtggccgtgctccaggtgagtccacctacgctaacctgccgatcgctgatttcggtgagaccaccactcgttaccacctcgacatggatgtggaagatcgcgtgggggttttggctgaattggctagcctgttctctgagcaaggaatctccctgcgtacaatccgacaggaagagcgcgatgatgatgcacgtctgatcgtggtcacccactctgcgctggaatctgatctttcccgcaccgttgaactgctgaaggctaagcctgttgttaaggcaatcaacagtgtgatccgcctcgaaagggactaattttactgacatggcaattgaactgaacgtcggtcgtaaggttaccgtcacggtacctggatcttctgcaaacctcggacctggctttgacactttaggtttggcactgtcggtatacgacactgtcgaagtggaaattattccatctggcttggaagtggaagtttttggcgaaggccaaggcgaagtccctcttgatggctcccacctggtggttaaagctattcgtgctggcctgaaggcagctgacgctgaagttcctggattgcgagtggtgtgccacaacaacattccgcagtctcgtggtcttggctcctctgctgcagcggcggttgctggtgttgctgcagctaatggtttggcggatttcccgctgactcaagagcagattgttcagttgtcctctgcctttgaaggccacccagataatgctgcggcttctgtgctgggtggagcagtggtgtcgtggacaaatctgtctatcgacggcaagagccagccacagtatgctgctgtaccacttgaggtgcaggacaatattcgtgcgactgcgctggttcctaatttccacgcatccaccgaagctgtgcgccgagtccttcccactgaagtcactcacatcgatgcgcgatttaacgtgtcccgcgttgcagtgatgatcgttgcgttgcagcagcgtcctgatttgctgtgggagggtactcgtgaccgtctgcaccagccttatcgtgcagaagtgttgcctattacctctgagtgggtaaaccgcctgcgcaaccgtggctacgcggcatacctttccggtgccggcccaaccgccatggtgctgtccactgagccaattccagacaaggttttggaagatgctcgtgagtctggcattaaggtgcttgagcttgaggttgcgggaccagtcaaggttgaagttaaccaaccttaggcccaacaaggaaggcccccttcgaatcaagaagggggccttattagtgcagcaattattcgctgaacacgtgaaccttacaggtgcccggcgcgttgagtggtttgagttccagctggatgcggttgttttcaccgaggctttcttggatgaatccggcgtggatggcgcagacgaaggctgatgggcgtttgtcgttg

SEQ ID NO: 6 - DNA, 1338 bp, Artificial Sequence
  T285I
atgacctcagcatctgccccaagctttaaccccggcaagggtcccggctcagcagtcggaattgcccttttaggattcggaacagtcggcactgaggtgatgcgtctgatgaccgagtacggtgatgaacttgcgcaccgcattggtggcccactggaggttcgtggcattgctgtttctgatatctcaaagccacgtgaaggcgttgcacctgagctgctcactgaggacgcttttgcactcatcgagcgcgaggatgttgacatcgtcgttgaggttatcggcggcattgagtacccacgtgaggtagttctcgcagctctgaaggccggcaagtctgttgttaccgccaataaggctcttgttgcagctcactctgctgagcttgctgatgcagcggaagccgcaaacgttgacctgtacttcgaggctgctgttgcaggcgcaattccagtggttggcccactgcgtcgctccctggctggcgatcagatccagtctgtgatgggcatcgttaacggcaccaccaacttcatcttggacgccatggattccaccggcgctgactatgcagattctttggctgaggcaactcgtttgggttacgccgaagctgatccaactgcagacgtcgaaggccatgacgccgcatccaaggctgcaattttggcatccatcgctttccacacccgtgttaccgcggatgatgtgtactgcgaaggtatcagcaacatcagcgctgccgacattgaggcagcacagcaggcaggccacaccatcaagttgttggccatctgtgagaagttcaccaacaaggaaggaaagtcggctatttctgctcgcgtgcacccgattctattacctgtgtcccacccactggcgtcggtaaacaagtcctttaatgcaatctttgttgaagcagaagcagctggtcgcctgatgttctacggaaacggtgcaggtggcgcgccaaccgcgtctgctgtgcttggcgacgtcgttggtgccgcacgaaacaaggtgcacggtggccgtgctccaggtgagtccacctacgctaacctgccgatcgctgatttcggtgagaccaccactcgttaccacctcgacatggatgtggaagatcgcgtgggggttttggctgaattggctagcctgttctctgagcaaggaatctccctgcgtacaatccgacaggaagagcgcgatgatgatgcacgtctgatcgtggtcacccactctgcgctggaatctgatctttcccgcaccgttgaactgctgaaggctaagcctgttgttaaggcaatcaacagtgtgatccgcctcgaaagggactaa

SEQ ID NO: 7 - DNA, 1338 bp, Artificial Sequence
  R398Q
atgacctcagcatctgccccaagctttaaccccggcaagggtcccggctcagcagtcggaattgcccttttaggattcggaacagtcggcactgaggtgatgcgtctgatgaccgagtacggtgatgaacttgcgcaccgcattggtggcccactggaggttcgtggcattgctgtttctgatatctcaaagccacgtgaaggcgttgcacctgagctgctcactgaggacgcttttgcactcatcgagcgcgaggatgttgacatcgtcgttgaggttatcggcggcattgagtacccacgtgaggtagttctcgcagctctgaaggccggcaagtctgttgttaccgccaataaggctcttgttgcagctcactctgctgagcttgctgatgcagcggaagccgcaaacgttgacctgtacttcgaggctgctgttgcaggcgcaattccagtggttggcccactgcgtcgctccctggctggcgatcagatccagtctgtgatgggcatcgttaacggcaccaccaacttcatcttggacgccatggattccaccggcgctgactatgcagattctttggctgaggcaactcgtttgggttacgccgaagctgatccaactgcagacgtcgaaggccatgacgccgcatccaaggctgcaattttggcatccatcgctttccacacccgtgttaccgcggatgatgtgtactgcgaaggtatcagcaacatcagcgctgccgacattgaggcagcacagcaggcaggccacaccatcaagttgttggccatctgtgagaagttcaccaacaaggaaggaaagtcggctatttctgctcgcgtgcacccgactctattacctgtgtcccacccactggcgtcggtaaacaagtcctttaatgcaatctttgttgaagcagaagcagctggtcgcctgatgttctacggaaacggtgcaggtggcgcgccaaccgcgtctgctgtgcttggcgacgtcgttggtgccgcacgaaacaaggtgcacggtggccgtgctccaggtgagtccacctacgctaacctgccgatcgctgatttcggtgagaccaccactcgttaccacctcgacatggatgtggaagatcgcgtgggggttttggctgaattggctagcctgttctctgagcaaggaatctccctgcgtacaatccaacaggaagagcgcgatgatgatgcacgtctgatcgtggtcacccactctgcgctggaatctgatctttcccgcaccgttgaactgctgaaggctaagcctgttgttaaggcaatcaacagtgtgatccgcctcgaaagggactaa

SEQ ID NO: 8 - DNA, 1338 bp, Artificial Sequence
  G378W
atgacctcagcatctgccccaagctttaaccccggcaagggtcccggctcagcagtcggaattgcccttttaggattcggaacagtcggcactgaggtgatgcgtctgatgaccgagtacggtgatgaacttgcgcaccgcattggtggcccactggaggttcgtggcattgctgtttctgatatctcaaagccacgtgaaggcgttgcacctgagctgctcactgaggacgcttttgcactcatcgagcgcgaggatgttgacatcgtcgttgaggttatcggcggcattgagtacccacgtgaggtagttctcgcagctctgaaggccggcaagtctgttgttaccgccaataaggctcttgttgcagctcactctgctgagcttgctgatgcagcggaagccgcaaacgttgacctgtacttcgaggctgctgttgcaggcgcaattccagtggttggcccactgcgtcgctccctggctggcgatcagatccagtctgtgatgggcatcgttaacggcaccaccaacttcatcttggacgccatggattccaccggcgctgactatgcagattctttggctgaggcaactcgtttgggttacgccgaagctgatccaactgcagacgtcgaaggccatgacgccgcatccaaggctgcaattttggcatccatcgctttccacacccgtgttaccgcggatgatgtgtactgcgaaggtatcagcaacatcagcgctgccgacattgaggcagcacagcaggcaggccacaccatcaagttgttggccatctgtgagaagttcaccaacaaggaaggaaagtcggctatttctgctcgcgtgcacccgactctattacctgtgtcccacccactggcgtcggtaaacaagtcctttaatgcaatctttgttgaagcagaagcagctggtcgcctgatgttctacggaaacggtgcaggtggcgcgccaaccgcgtctgctgtgcttggcgacgtcgttggtgccgcacgaaacaaggtgcacggtggccgtgctccaggtgagtccacctacgctaacctgccgatcgctgatttcggtgagaccaccactcgttaccacctcgacatggatgtggaagatcgcgtgtgggttttggctgaattggctagcctgttctctgagcaaggaatctccctgcgtacaatccgacaggaagagcgcgatgatgatgcacgtctgatcgtggtcacccactctgcgctggaatctgatctttcccgcaccgttgaactgctgaaggctaagcctgttgttaaggcaatcaacagtgtgatccgcctcgaaagggactaa

SEQ ID NO: 9 - DNA, 1338 bp, Artificial Sequence
  G378S
atgacctcagcatctgccccaagctttaaccccggcaagggtcccggctcagcagtcggaattgcccttttaggattcggaacagtcggcactgaggtgatgcgtctgatgaccgagtacggtgatgaacttgcgcaccgcattggtggcccactggaggttcgtggcattgctgtttctgatatctcaaagccacgtgaaggcgttgcacctgagctgctcactgaggacgcttttgcactcatcgagcgcgaggatgttgacatcgtcgttgaggttatcggcggcattgagtacccacgtgaggtagttctcgcagctctgaaggccggcaagtctgttgttaccgccaataaggctcttgttgcagctcactctgctgagcttgctgatgcagcggaagccgcaaacgttgacctgtacttcgaggctgctgttgcaggcgcaattccagtggttggcccactgcgtcgctccctggctggcgatcagatccagtctgtgatgggcatcgttaacggcaccaccaacttcatcttggacgccatggattccaccggcgctgactatgcagattctttggctgaggcaactcgtttgggttacgccgaagctgatccaactgcagacgtcgaaggccatgacgccgcatccaaggctgcaattttggcatccatcgctttccacacccgtgttaccgcggatgatgtgtactgcgaaggtatcagcaacatcagcgctgccgacattgaggcagcacagcaggcaggccacaccatcaagttgttggccatctgtgagaagttcaccaacaaggaaggaaagtcggctatttctgctcgcgtgcacccgactctattacctgtgtcccacccactggcgtcggtaaacaagtcctttaatgcaatctttgttgaagcagaagcagctggtcgcctgatgttctacggaaacggtgcaggtggcgcgccaaccgcgtctgctgtgcttggcgacgtcgttggtgccgcacgaaacaaggtgcacggtggccgtgctccaggtgagtccacctacgctaacctgccgatcgctgatttcggtgagaccaccactcgttaccacctcgacatggatgtggaagatcgcgtgagcgttttggctgaattggctagcctgttctctgagcaaggaatctccctgcgtacaatccgacaggaagagcgcgatgatgatgcacgtctgatcgtggtcacccactctgcgctggaatctgatctttcccgcaccgttgaactgctgaaggctaagcctgttgttaaggcaatcaacagtgtgatccgcctcgaaagggactaa

SEQ ID NO: 10 - protein, 445 aa, Artificial Sequence
  Hom (KFCC10881-1)
MTSASAPSFNPGKGPGSAVGIALLGFGTVGTEVMRLMTEYGDELAHRIGGPLEVRGIAVSDISKPREGVAPELLTEDAFALIEREDVDIVVEVIGGIEYPREVVLAALKAGKSVVTANKALVAAHSAELADAAEAANVDLYFEAAVAGAIPVVGPLRRSLAGDQIQSVMGIVNGTTNFILDAMDSTGADYADSLAEATRLGYAEADPTADVEGHDAASKAAILASIAFHTRVTADDVYCEGISNISAADIEAAQQAGHTIKLLAICEKFTNKEGKSAISARVHPILLPVSHPLASVNKSFNAIFVEAEAAGRLMFYGNGAGGAPTASAVLGDVVGAARNKVHGGRAPGESTYANLPIADFGETTTRYHLDMDVEDRVGVLAELASLFSEQGISLRTIRQEERDDDARLIVVTHSALESDLSRTVELLKAKPVVKAINSVIRLERD

SEQ ID NO: 11 - protein, 445 aa, Artificial Sequence
  Hom (KFCC10881-14)
MTSASAPSFNPGKGPGSAVGIALLGFGTVGTEVMRLMTEYGDELAHRIGGPLEVRGIAVSDISKPREGVAPELLTEDAFALIEREDVDIVVEVIGGIEYPREVVLAALKAGKSVVTANKALVAAHSAELADAAEAANVDLYFEAAVAGAIPVVGPLRRSLAGDQIQSVMGIVNGTTNFILDAMDSTGADYADSLAEATRLGYAEADPTADVEGHDAASKAAILASIAFHTRVTADDVYCEGISNISAADIEAAQQAGHTIKLLAICEKFTNKEGKSAISARVHPTLLPVSHPLASVNKSFNAIFVEAEAAGRLMFYGNGAGGAPTASAVLGDVVGAARNKVHGGRAPGESTYANLPIADFGETTTRYHLDMDVEDRVGVLAELASLFSEQGISLRTIQQEERDDDARLIVVTHSALESDLSRTVELLKAKPVVKAINSVIRLERD

SEQ ID NO: 12 - protein, 445 aa, Artificial Sequence
  Hom (KFCC10881-19)
MTSASAPSFNPGKGPGSAVGIALLGFGTVGTEVMRLMTEYGDELAHRIGGPLEVRGIAVSDISKPREGVAPELLTEDAFALIEREDVDIVVEVIGGIEYPREVVLAALKAGKSVVTANKALVAAHSAELADAAEAANVDLYFEAAVAGAIPVVGPLRRSLAGDQIQSVMGIVNGTTNFILDAMDSTGADYADSLAEATRLGYAEADPTADVEGHDAASKAAILASIAFHTRVTADDVYCEGISNISAADIEAAQQAGHTIKLLAICEKFTNKEGKSAISARVHPTLLPVSHPLASVNKSFNAIFVEAEAAGRLMFYGNGAGGAPTASAVLGDVVGAARNKVHGGRAPGESTYANLPIADFGETTTRYHLDMDVEDRVWVLAELASLFSEQGISLRTIRQEERDDDARLIVVTHSALESDLSRTVELLKAKPVVKAINSVIRLERD

SEQ ID NO: 13 - protein, 445 aa, Artificial Sequence
  Hom (KFCC10881-22)
MTSASAPSFNPGKGPGSAVGIALLGFGTVGTEVMRLMTEYGDELAHRIGGPLEVRGIAVSDISKPREGVAPELLTEDAFALIEREDVDIVVEVIGGIEYPREVVLAALKAGKSVVTANKALVAAHSAELADAAEAANVDLYFEAAVAGAIPVVGPLRRSLAGDQIQSVMGIVNGTTNFILDAMDSTGADYADSLAEATRLGYAEADPTADVEGHDAASKAAILASIAFHTRVTADDVYCEGISNISAADIEAAQQAGHTIKLLAICEKFTNKEGKSAISARVHPTLLPVSHPLASVNKSFNAIFVEAEAAGRLMFYGNGAGGAPTASAVLGDVVGAARNKVHGGRAPGESTYANLPIADFGETTTRYHLDMDVEDRVSVLAELASLFSEQGISLRTIRQEERDDDARLIVVTHSALESDLSRTVELLKAKPVVKAINSVIRLERD

SEQ ID NO: 14 - DNA, 34 bp, Artificial Sequence
  primer
tcgagctcggtacccctgcgacagcatggaactc

SEQ ID NO: 15 - DNA, 34 bp, Artificial Sequence
  primer
ctctagaggatccccttagtccctttcgaggcgg

SEQ ID NO: 16 - DNA, 18 bp, Artificial Sequence
  primer
caccggcgctgactatgc

SEQ ID NO: 17 - DNA, 18 bp, Artificial Sequence
  primer
aatcgggtgcacgcgagc

SEQ ID NO: 18 - DNA, 18 bp, Artificial Sequence
  primer
ttggattgtacgcaggga

SEQ ID NO: 19 - DNA, 18 bp, Artificial Sequence
  primer
ccacacgcgatcttccac

SEQ ID NO: 20 - DNA, 18 bp, Artificial Sequence
  primer
gctcacgcgatcttccac

SEQ ID NO: 21 - DNA, 18 bp, Artificial Sequence
  primer
ttagtccctttcgaggcg

SEQ ID NO: 22 - protein, 421 aa, Artificial Sequence
  lysC(L377K)
VALVVQKYGGSSLESAERIRNVAERIVATKKAGNDVVVVCSAMGDTTDELLELAAAVNPVPPAREMDMLLTAGERISNALVAMAIESLGAEAQSFTGSQAGVLTTERHGNARIVDVTPGRVREALDEGKICIVAGFQGVNKETRDVTTLGRGGSDTTAVALAAALNADVCEIYSDVDGVYTADPRIVPNAQKLEKLSFEEMLELAAVGSKILVLRSVEYARAFNVPLRVRSSYSNDPGTLIAGSMEDIPVEEAVLTGVATDKSEAKVTVLGISDKPGEAAKVFRALADAEINIDMVLQNVSSVEDGTTDITFTCPRSDGRRAMEILKKLQVQGNWTNVLYDDQVGKVSLVGAGMKSHPGVTAEFMEALRDVNVNIEKISTSEIRISVLIREDDLDAAARALHEQFQLGGEDEAVVYAGTGR

SEQ ID NO: 23 - DNA, 34 bp, Artificial Sequence
  primer
tcgagctcggtacccgctgcgcagtgttgaatac

SEQ ID NO: 24 - DNA, 30 bp, Artificial Sequence
  primer
tggaaatcttttcgatgttcacgttgacat

SEQ ID NO: 25 - DNA, 30 bp, Artificial Sequence
  primer
atgtcaacgtgaacatcgaaaagatttcca

SEQ ID NO: 26 - DNA, 34 bp, Artificial Sequence
  primer
ctctagaggatccccgttcacctcagagacgatt

SEQ ID NO: 27 - DNA, 28 bp, Artificial Sequence
  primer
acggatcccagactccaaagcaaaagcg

SEQ ID NO: 28 - DNA, 30 bp, Artificial Sequence
  primer
acaccacggcagaaccaggtgcaaaggaca

SEQ ID NO: 29 - DNA, 30 bp, Artificial Sequence
  primer
ctggttctgccgtggtgtgcatcatctctg

SEQ ID NO: 30 - DNA, 28 bp, Artificial Sequence
  primer
acggatccaaccaaacttgctcacactc

SEQ ID NO: 31 - DNA, 1161 bp, Artificial Sequence
  metB gene
ttgtcttttgacccaaacacccagggtttctccactgcatcgattcacgctgggtatgagccagacgactactacggttcgattaacaccccaatctatgcctccaccaccttcgcgcagaacgctccaaacgaactgcgcaaaggctacgagtacacccgtgtgggcaaccccaccatcgtggcattagagcagaccgtcgcagcactcgaaggcgcaaagtatggccgcgcattctcctccggcatggctgcaaccgacatcctgttccgcatcatcctcaagccgggcgatcacatcgtcctcggcaacgatgcttacggcggaacctaccgcctgatcgacaccgtattcaccgcatggggcgtcgaatacaccgttgttgatacctccgtcgtggaagaggtcaaggcagcgatcaaggacaacaccaagctgatctgggtggaaaccccaaccaacccagcacttggcatcaccgacatcgaagcagtagcaaagctcaccgaaggcaccaacgccaagctggttgttgacaacaccttcgcatccccatacctgcagcagccactaaaactcggcgcacacgcagtcctgcactccaccaccaagtacatcggaggacactccgacgttgttggcggccttgtggttaccaacgaccaggaaatggacgaagaactgctgttcatgcagggcggcatcggaccgatcccatcagttttcgatgcatacctgaccgcccgtggcctcaagacccttgcagtgcgcatggatcgccactgcgacaacgcagaaaagatcgcggaattcctggactcccgcccagaggtctccaccgtgctctacccaggtctgaagaaccacccaggccacgaagtcgcagcgaagcagatgaagcgcttcggcggcatgatctccgtccgtttcgcaggcggcgaagaagcagctaagaagttctgtacctccaccaaactgatctgtctggccgagtccctcggtggcgtggaatccctcctggagcacccagcaaccatgacccaccagtcagctgccggctctcagctcgaggttccccgcgacctcgtgcgcatctccattggtattgaagacattgaagacctgctcgcagatgtcgagcaggccctcaataacctttag

SEQ ID NO: 32 - DNA, 24 bp, Artificial Sequence
  primer
tctagacgcccgcatactggcttc

SEQ ID NO: 33 - DNA, 37 bp, Artificial Sequence
  primer
cccatccactaaacttaaacagatgtgatcgcccggc

SEQ ID NO: 34 - DNA, 38 bp, Artificial Sequence
  primer
tgtttaagtttagtggatggggaagaaccacccaggcc

SEQ ID NO: 35 - DNA, 23 bp, Artificial Sequence
  primer
gtcgaccaatcgtccagagggcg

SEQ ID NO: 36 - DNA, 1314 bp, Artificial Sequence
  metY gene
atgccaaagtacgacaattccaatgctgaccagtggggctttgaaacccgctccattcacgcaggccagtcagtagacgcacagaccagcgcacgaaaccttccgatctaccaatccaccgctttcgtgttcgactccgctgagcacgccaagcagcgtttcgcacttgaggatctaggccctgtttactcccgcctcaccaacccaaccgttgaggctttggaaaaccgcatcgcttccctcgaaggtggcgtccacgctgtagcgttctcctccggacaggccgcaaccaccaacgccattttgaacctggcaggagcgggcgaccacatcgtcacctccccacgcctctacggtggcaccgagactctattccttatcactcttaaccgcctgggtatcgatgtttccttcgtggaaaaccccgacgaccctgagtcctggcaggcagccgttcagccaaacaccaaagcattcttcggcgagactttcgccaacccacaggcagacgtcctggatattcctgcggtggctgaagttgcgcaccgcaacagcgttccactgatcatcgacaacaccatcgctaccgcagcgctcgtgcgcccgctcgagctcggcgcagacgttgtcgtcgcttccctcaccaagttctacaccggcaacggctccggactgggcggcgtgcttatcgacggcggaaagttcgattggactgtcgaaaaggatggaaagccagtattcccctacttcgtcactccagatgctgcttaccacggattgaagtacgcagaccttggtgcaccagccttcggcctcaaggttcgcgttggccttctacgcgacaccggctccaccctctccgcattcaacgcatgggctgcagtccagggcatcgacaccctttccctgcgcctggagcgccacaacgaaaacgccatcaaggttgcagaattcctcaacaaccacgagaaggtggaaaaggttaacttcgcaggcctgaaggattccccttggtacgcaaccaaggaaaagcttggcctgaagtacaccggctccgttctcaccttcgagatcaagggcggcaaggatgaggcttgggcatttatcgacgccctgaagctacactccaaccttgcaaacatcggcgatgttcgctccctcgttgttcacccagcaaccaccacccattcacagtccgacgaagctggcctggcacgcgcgggcgttacccagtccaccgtccgcctgtccgttggcatcgagaccattgatgatatcatcgctgacctcgaaggcggctttgctgcaatctag

SEQ ID NO: 37 - DNA, 24 bp, Artificial Sequence
  primer
tctagaccatcctgcaccatttag

SEQ ID NO: 38 - DNA, 37 bp, Artificial Sequence
  primer
cccatccactaaacttaaacacgctcctgccaggttc

SEQ ID NO: 39 - DNA, 39 bp, Artificial Sequence
  primer
tgtttaagtttagtggatgggcttggtacgcaaccaagg

SEQ ID NO: 40 - DNA, 23 bp, Artificial Sequence
  primer
gtcgacgattgctccggcttcgg

SEQ ID NO: 41 - DNA, 2213 bp, Artificial Sequence
  mcbR gene
aatctggatttccgccaggttttggcacgcccgtctggtttaggcaatgagataccgaacacacgtgccaaaagttcggctttttcgccgatcttgtcacgcctgcctggtttgtcttgtaaagagtgatttcatggccgagactcctaaaagtttgacctcacaggattgcttctaagggcctctccaatctccactgaggtacttaatccttccggggaattcgggcgcttaaatcgagaaattaggccatcaccttttaataacaatacaatgaataattggaataggtcgacacctttggagcggagccggttaaaattggcagcattcaccgaaagaaaaggagaaccacatgcttgccctaggttggattacatggatcattattggtggtctagctggttggattgcctccaagattaaaggcactgatgctcagcaaggaattttgctgaacatagtcgtcggtattatcggtggtttgttaggcggctggctgcttggaatcttcggagtggatgttgccggtggcggcttgatcttcagcttcatcacatgtctgattggtgctgtcattttgctgacgatcgtgcagttcttcactcggaagaagtaatctgctttaaatccgtagggcctgttgatatttcgatatcaacaggccttttggtcattttggggtggaaaaagcgctagacttgcctgtggattaaaactatacgaaccggtttgtctatattggtgttagacagttcgtcgtatcttgaaacagaccaacccgaaaggacgtggccgaacgtggctgctagcgcttcaggcaagagtaaaacaagtgccggggcaaaccgtcgtcgcaatcgaccaagcccccgacagcgtctcctcgatagcgcaaccaaccttttcaccacagaaggtattcgcgtcatcggtattgatcgtatcctccgtgaagctgacgtggcgaaggcgagcctctattcccttttcggatcgaaggacgccttggttattgcatacctggagaacctcgatcagctgtggcgtgaagcgtggcgtgagcgcaccgtcggtatgaaggatccggaagataaaatcatcgcgttctttgatcagtgcattgaggaagaaccagaaaaagatttccgcggctcgcactttcagaatgcggctagtgagtaccctcgccccgaaactgatagcgaaaagggcattgttgcagcagtgttagagcaccgcgagtggtgtcataagactctgactgatttgctcactgagaagaacggctacccaggcaccacccaggcgaatcagctgttggtgttccttgatggtggacttgctggatctcgattggtccacaacatcagtcctcttgagacggctcgcgatttggctcggcagttgttgtcggctccacctgcggactactcaatttagtttcttcattttccgaaggggtatcttcgttgggggaggcgtcgataagccccttctttttagctttaacctcagcgcgacgctgctttaagcgctgcatggcggcgcggttcatttcacgttgcgtttcgcgcctcttgttcgcgatttctttgcgggcctgttttgcttcgttgatttcggcagtacgggttttggtgagttccacgtttgttgcgtgaagcgttgaggcgttccatggggtgagaatcatcagggcgcggtttttgcgtcgtgtccacaggaagatgcgcttttctttttgttttgcgcggtagatgtcgcgctgctctaggtggtgcactttgaaatcgtcggtaagtgggtatttgcgttccaaaatgaccatcatgatgattgtttggaggagcgtccacaggttgttgctgacccaatagagtgcgattgctgtggggaatggtcctgtgaggccaagggacagtgggaagatcggcgcgaggatcgacatcacgatcatgaacttcagcatgccgttagagaatccggatgcgtaatcgttggtttggaagctgcggtacatggacatcgccatgttgattgcggtgaggattgcggctgtgatgaacagtggcaaaacgaaactaagaacttccgcctgcgtggtgctcaaatattttagctgctcagtgggcatcgaaacataagcgggcagaggcacattgctcacgcgaccagcgaggaaagattccacttcctcaggagttaggaag

SEQ ID NO: 42 - DNA, 28 bp, Artificial Sequence
  primer
ggcccgggcctgcctggtttgtcttgta

SEQ ID NO: 43 - DNA, 35 bp, Artificial Sequence
  primer
cggaaaatgaagaaagttcggccacgtcctttcgg

SEQ ID NO: 44 - DNA, 35 bp, Artificial Sequence
  primer
aggacgtggccgaactttcttcattttccgaaggg

SEQ ID NO: 45 - DNA, 28 bp, Artificial Sequence
  primer
atcccggggtttcgatgcccactgagca

SEQ ID NO: 46 - DNA, 20 bp, Artificial Sequence
  primer
aatctggatttccgccaggt

SEQ ID NO: 47 - DNA, 20 bp, Artificial Sequence
  primer
cttcctaactcctgaggaag

SEQ ID NO: 48 - DNA, 1338 bp, Artificial Sequence
  wild-type hom gene
atgacctcagcatctgccccaagctttaaccccggcaagggtcccggctcagcagtcggaattgcccttttaggattcggaacagtcggcactgaggtgatgcgtctgatgaccgagtacggtgatgaacttgcgcaccgcattggtggcccactggaggttcgtggcattgctgtttctgatatctcaaagccacgtgaaggcgttgcacctgagctgctcactgaggacgcttttgcactcatcgagcgcgaggatgttgacatcgtcgttgaggttatcggcggcattgagtacccacgtgaggtagttctcgcagctctgaaggccggcaagtctgttgttaccgccaataaggctcttgttgcagctcactctgctgagcttgctgatgcagcggaagccgcaaacgttgacctgtacttcgaggctgctgttgcaggcgcaattccagtggttggcccactgcgtcgctccctggctggcgatcagatccagtctgtgatgggcatcgttaacggcaccaccaacttcatcttggacgccatggattccaccggcgctgactatgcagattctttggctgaggcaactcgtttgggttacgccgaagctgatccaactgcagacgtcgaaggccatgacgccgcatccaaggctgcaattttggcatccatcgctttccacacccgtgttaccgcggatgatgtgtactgcgaaggtatcagcaacatcagcgctgccgacattgaggcagcacagcaggcaggccacaccatcaagttgttggccatctgtgagaagttcaccaacaaggaaggaaagtcggctatttctgctcgcgtgcacccgactctattacctgtgtcccacccactggcgtcggtaaacaagtcctttaatgcaatctttgttgaagcagaagcagctggtcgcctgatgttctacggaaacggtgcaggtggcgcgccaaccgcgtctgctgtgcttggcgacgtcgttggtgccgcacgaaacaaggtgcacggtggccgtgctccaggtgagtccacctacgctaacctgccgatcgctgatttcggtgagaccaccactcgttaccacctcgacatggatgtggaagatcgcgtgggggttttggctgaattggctagcctgttctctgagcaaggaatctccctgcgtacaatccgacaggaagagcgcgatgatgatgcacgtctgatcgtggtcacccactctgcgctggaatctgatctttcccgcaccgttgaactgctgaaggctaagcctgttgttaaggcaatcaacagtgtgatccgcctcgaaagggactaa

SEQ ID NO: 49 - protein, 445 aa, Artificial Sequence; identical to SEQ ID NO: 1
  ATCC14067 hom (NCgl1136)

SEQ ID NO: 50 - protein, 445 aa, Artificial Sequence
  ATCC13869 hom
MTSASAPSFNPGKGPGSAVGIALLGFGTVGTEVMRLMTEYGDELAHRIGGPLEVRGIAVSDISKPREGVAPELLTEDAFALIEREDVDIVVEVIGGIEYPREVVLAALKAGKSVVTANKALVAAHSAELADAAEAANVDLYFEAAVAAAIPVVGPLRRSLAGDQIQSVMGIVNGTTNFILDAMDSTGADYADSLAEATRLGYAEADPTADVEGHDAASKAAILASIAFHTRVTADDVYCEGISNISAADIEAAQQAGHTIKLLAICEKFTNKEGKSAISARVHPTLLPVSHPLASVNKSFNAIFVEAEAAGRLMFYGNGAGGAPTASAVLGDVVGAARNKVHGGRAPGESTYANLPIADFGETTTRYHLDMDVEDRVGVLAELASLFSEQGISLRTIRQEERDDDARLIVVTHSALESDLSRTVELLKAKPVVKAINSVIRLERD